European Patent Specification EP 3 430 132 B1, published April 30, 2025. Title: Generation Of Midbrain-Specific Organoids From Human Pluripotent Stem Cells. Applicant: Agency for Science, Technology and Research. The sequence listing filed with the application follows.

SEQUENCE LISTING (112 sequences)

SEQ ID NO: 1 - DNA, 24 bp, Artificial sequence
  GAPDH forward primer
caagatcatcagcaatgcctcctg

SEQ ID NO: 2 - DNA, 22 bp, Artificial sequence
  GAPDH reverse primer
gcctgcttcaccaccttcttga

SEQ ID NO: 3 - DNA, 20 bp, Artificial sequence
  OCT4 forward primer
gtggaggaagctgacaacaa

SEQ ID NO: 4 - DNA, 20 bp, Artificial sequence
  OCT4 reverse primer
attctccaggttgcctctca

SEQ ID NO: 5 - DNA, 21 bp, Artificial sequence
  NANOG forward primer
tttgtgggcctgaagaaaact

SEQ ID NO: 6 - DNA, 21 bp, Artificial sequence
  NANOG reverse primer
agggctgtcctgaataagcag

SEQ ID NO: 7 - DNA, 21 bp, Artificial sequence
  PAX6 forward primer
tccacccggcagaagattgta

SEQ ID NO: 8 - DNA, 21 bp, Artificial sequence
  PAX6 reverse primer
tgtctcggatttcccaagcaa

SEQ ID NO: 9 - DNA, 21 bp, Artificial sequence
  SOX1 forward primer
gaacgccttcatggtgtggtc

SEQ ID NO: 10 - DNA, 21 bp, Artificial sequence
  SOX1 reverse primer
tgtaatccgggtgctccttca

SEQ ID NO: 11 - DNA, 21 bp, Artificial sequence
  OTX2 forward primer
ccagacatcttcatgcgagag

SEQ ID NO: 12 - DNA, 21 bp, Artificial sequence
  OTX2 reverse primer
ggcaggtctcactttgttttg

SEQ ID NO: 13 - DNA, 20 bp, Artificial sequence
  CORIN forward primer
aatcccacaacagagcatcg

SEQ ID NO: 14 - DNA, 20 bp, Artificial sequence
  CORIN reverse primer
ggagcagttgacctcgtcag

SEQ ID NO: 15 - DNA, 20 bp, Artificial sequence
  FOXA2 forward primer
ggggtagtgcatcacctgtt

SEQ ID NO: 16 - DNA, 20 bp, Artificial sequence
  FOXA2 reverse primer
ccgttctccatcaacaacct

SEQ ID NO: 17 - DNA, 19 bp, Artificial sequence
  MAP2 forward primer
cgaagcgccaatggattcc

SEQ ID NO: 18 - DNA, 22 bp, Artificial sequence
  MAP2 reverse primer
tgaactatccttgcagacacct

SEQ ID NO: 19 - DNA, 22 bp, Artificial sequence
  TH forward primer
tgtctgaggagcctgagattcg

SEQ ID NO: 20 - DNA, 20 bp, Artificial sequence
  TH reverse primer
gcttgtccttggcgtcactg

SEQ ID NO: 21 - DNA, 20 bp, Artificial sequence
  PITX3 forward primer
ccaaccttagtccgtgccag

SEQ ID NO: 22 - DNA, 20 bp, Artificial sequence
  PITX3 reverse primer
tgtgtagggcctagtccacc

SEQ ID NO: 23 - DNA, 20 bp, Artificial sequence
  EN1 forward primer
tctcgctgtctctccctctc

SEQ ID NO: 24 - DNA, 20 bp, Artificial sequence
  EN1 reverse primer
cgtggcttactccccattta

SEQ ID NO: 25 - DNA, 19 bp, Artificial sequence
  EN2 forward primer
ccggcgtgggtctactgta

SEQ ID NO: 26 - DNA, 22 bp, Artificial sequence
  EN2 reverse primer
cctctttgttcgggttcttctt

SEQ ID NO: 27 - DNA, 20 bp, Artificial sequence
  NURR1 forward primer
gctggactccccattgcttt

SEQ ID NO: 28 - DNA, 20 bp, Artificial sequence
  NURR1 reverse primer
cggagctgtattctcccgaa

SEQ ID NO: 29 - DNA, 21 bp, Artificial sequence
  LMX1A forward primer
acgtccgagaaccatcttgac

SEQ ID NO: 30 - DNA, 19 bp, Artificial sequence
  LMX1A reverse primer
caccaccgtttgtctgagc

SEQ ID NO: 31 - DNA, 19 bp, Artificial sequence
  LMX1B forward primer
cggactgcgccaagatgtt

SEQ ID NO: 32 - DNA, 20 bp, Artificial sequence
  LMX1B reverse primer
ttgactcgcatcaggaagcg

SEQ ID NO: 33 - DNA, 21 bp, Artificial sequence
  DDC forward primer
attcatctgccctgagttccg

SEQ ID NO: 34 - DNA, 21 bp, Artificial sequence
  DDC reverse primer
ccaatagccatttgtggggat

SEQ ID NO: 35 - DNA, 20 bp, Artificial sequence
  ALDH1A1 forward primer
ccgtggcgtactatggatgc

SEQ ID NO: 36 - DNA, 22 bp, Artificial sequence
  ALDH1A1 reverse primer
gcagcagacgatctctttcgat

SEQ ID NO: 37 - DNA, 22 bp, Artificial sequence
  ALDH1A2 forward primer
gggtgtgttcttcaatcaaggt

SEQ ID NO: 38 - DNA, 19 bp, Artificial sequence
  ALDH1A2 reverse primer
tggtggggtcaaagggact

SEQ ID NO: 39 - DNA, 20 bp, Artificial sequence
  GIRK2 forward primer
cacatcagccgagatcggac

SEQ ID NO: 40 - DNA, 21 bp, Artificial sequence
  GIRK2 reverse primer
ggtagcgataggtctccctca

SEQ ID NO: 41 - DNA, 21 bp, Artificial sequence
  KCNS3 forward primer
aggagctgtgcgtattctcat

SEQ ID NO: 42 - DNA, 21 bp, Artificial sequence
  KCNS3 reverse primer
cttgcgttcctggtagcgatt

SEQ ID NO: 43 - DNA, 19 bp, Artificial sequence
  SOX6 forward primer
agggagtcttgccgatgtg

SEQ ID NO: 44 - DNA, 22 bp, Artificial sequence
  SOX6 reverse primer
caggctctcaggtgtaccttta

SEQ ID NO: 45 - DNA, 23 bp, Artificial sequence
  OXR1 forward primer
ttcgaccaaacctaagtgatccc

SEQ ID NO: 46 - DNA, 22 bp, Artificial sequence
  OXR1 reverse primer
ggggtgtctaaacctgtcattg

SEQ ID NO: 47 - DNA, 20 bp, Artificial sequence
  SNCG forward primer
tgagcagcgtcaacactgtg

SEQ ID NO: 48 - DNA, 20 bp, Artificial sequence
  SNCG reverse primer
gaggtgaccgcgatgttctc

SEQ ID NO: 49 - DNA, 23 bp, Artificial sequence
  SATB1 forward primer
agagctgtcagtggaaggaaaca

SEQ ID NO: 50 - DNA, 24 bp, Artificial sequence
  SATB1 reverse primer
gtggcactgttgaacgaaacaaat

SEQ ID NO: 51 - DNA, 19 bp, Artificial sequence
  ZDHHC2 forward primer
tcccggtggtgttcatcac

SEQ ID NO: 52 - DNA, 22 bp, Artificial sequence
  ZDHHC2 reverse primer
caacttgttcgccagtgttttc

SEQ ID NO: 53 - DNA, 19 bp, Artificial sequence
  RAB3C forward primer
ggaagacgagcgggtcatc

SEQ ID NO: 54 - DNA, 23 bp, Artificial sequence
  RAB3C reverse primer
ctctctgacattttgtcgcagat

SEQ ID NO: 55 - DNA, 21 bp, Artificial sequence
  FGF1 forward primer
acaccgacgggcttttatacg

SEQ ID NO: 56 - DNA, 21 bp, Artificial sequence
  FGF1 reverse primer
cccattcttcttgaggccaac

SEQ ID NO: 57 - DNA, 21 bp, Artificial sequence
  GAD1 forward primer
gcggaccccaataccactaac

SEQ ID NO: 58 - DNA, 21 bp, Artificial sequence
  GAD1 reverse primer
cacaaggcgactcttctcttc

SEQ ID NO: 59 - DNA, 22 bp, Artificial sequence
  CALB1 foward primer
tgtggatcagtatgggcaaaga

SEQ ID NO: 60 - DNA, 23 bp, Artificial sequence
  CALB1 reverse primer
ctcagtttctatgaagccactgt

SEQ ID NO: 61 - DNA, 19 bp, Artificial sequence
  CALB2 forward primer
agcgccgagtttatggagg

SEQ ID NO: 62 - DNA, 21 bp, Artificial sequence
  CALB2 reverse primer
tggtttgggtgtattcctgga

SEQ ID NO: 63 - DNA, 19 bp, Artificial sequence
  TACR3 forward primer
ctctggtccctggcgtatg

SEQ ID NO: 64 - DNA, 22 bp, Artificial sequence
  TACR3 reverse primer
tgaagcgcgtagatgaaattga

SEQ ID NO: 65 - DNA, 20 bp, Artificial sequence
  CARTPT forward primer
ccgagccctggacatctact

SEQ ID NO: 66 - DNA, 23 bp, Artificial sequence
  CARTPT reverse primer
atgggaacacgtttactcttgag

SEQ ID NO: 67 - DNA, 20 bp, Artificial sequence
  VGF forward primer
cgctgacccgagtgaatctg

SEQ ID NO: 68 - DNA, 19 bp, Artificial sequence
  VGF reverse primer
catacgcgcctggaattga

SEQ ID NO: 69 - DNA, 24 bp, Artificial sequence
  VIP forward primer
ccaaaacaaaccagaacagtcagc

SEQ ID NO: 70 - DNA, 23 bp, Artificial sequence
  VIP reverse primer
tgagaagagtcaggagcacaagg

SEQ ID NO: 71 - DNA, 21 bp, Artificial sequence
  LPL forward primer
tcattcccggagtagcagagt

SEQ ID NO: 72 - DNA, 19 bp, Artificial sequence
  LPL reverse primer
ggccacaagttttggcacc

SEQ ID NO: 73 - DNA, 21 bp, Artificial sequence
  EFNB3 forward primer
ctcggcgaataagaggttcca

SEQ ID NO: 74 - DNA, 20 bp, Artificial sequence
  EFNB3 reverse primer
gtgaagcggagatccaggtc

SEQ ID NO: 75 - DNA, 19 bp, Artificial sequence
  EGR1 forward primer
ggtcagtggcctagtgagc

SEQ ID NO: 76 - DNA, 20 bp, Artificial sequence
  EGR1 reverse primer
gtgccgctgagtaaatggga

SEQ ID NO: 77 - DNA, 23 bp, Artificial sequence
  FZD1 forward primer
atcgaagccaactcacagtattt

SEQ ID NO: 78 - DNA, 19 bp, Artificial sequence
  FZD1 reverse primer
cacgttgttaagccccacg

SEQ ID NO: 79 - DNA, 19 bp, Artificial sequence
  ADCYAP1 forward primer
ccactcggacgggatcttc

SEQ ID NO: 80 - DNA, 22 bp, Artificial sequence
  ADCYAP1 reverse primer
gccgccaagtatttcttgacag

SEQ ID NO: 81 - DNA, 21 bp, Artificial sequence
  SDC2 forward primer
tggaaaccacgacgctgaata

SEQ ID NO: 82 - DNA, 22 bp, Artificial sequence
  SDC2 reverse primer
ataactccaccagcaatgacag

SEQ ID NO: 83 - DNA, 22 bp, Artificial sequence
  NEFM forward primer
gaaatcgctgcgtacagaaaac

SEQ ID NO: 84 - DNA, 21 bp, Artificial sequence
  NEFM reverse primer
taatggctgtcagggcctctt

SEQ ID NO: 85 - DNA, 23 bp, Artificial sequence
  LRRK2 forward primer
ttttgatgccatgcactcatttc

SEQ ID NO: 86 - DNA, 23 bp, Artificial sequence
  LRRK2 reverse primer
ggaatcgctagggaatgtaaaca

SEQ ID NO: 87 - DNA, 21 bp, Artificial sequence
  PARK2 forward primer
cccacctctgacaaggaaaca

SEQ ID NO: 88 - DNA, 21 bp, Artificial sequence
  PARK2 reverse primer
tcgtgaacaaactgccgatca

SEQ ID NO: 89 - DNA, 19 bp, Artificial sequence
  PARK7 forward primer
aaccggaagggcctgatag

SEQ ID NO: 90 - DNA, 21 bp, Artificial sequence
  PARK7 reverse primer
gcaagagggtgtgttgtaact

SEQ ID NO: 91 - DNA, 23 bp, Artificial sequence
  SNCA forward primer
aagagggtgttctctatgtaggc

SEQ ID NO: 92 - DNA, 22 bp, Artificial sequence
  SNCA reverse primer
gctcctccaacatttgtcactt

SEQ ID NO: 93 - DNA, 21 bp, Artificial sequence
  NCAM forward primer
ggctccttggactcatctttc

SEQ ID NO: 94 - DNA, 21 bp, Artificial sequence
  NCAM reverse primer
gacatcacctgctacttcctg

SEQ ID NO: 95 - DNA, 23 bp, Artificial sequence
  MAPT forward primer
gaagattgggtccctggacaata

SEQ ID NO: 96 - DNA, 20 bp, Artificial sequence
  MAPT reverse primer
aggtcagcttgtgggtttca

SEQ ID NO: 97 - DNA, 24 bp, Artificial sequence
  GAD2 forward primer
caaacatttatcaacatgcgcttc

SEQ ID NO: 98 - DNA, 21 bp, Artificial sequence
  GAD2 reverse primer
ctatgacactggagacaaggc

SEQ ID NO: 99 - DNA, 22 bp, Artificial sequence
  VGAT forward primer
agatgatgagaaacaaccccag

SEQ ID NO: 100 - DNA, 20 bp, Artificial sequence
  VGAT reverse primer
cacgacaagcccaaaatcac

SEQ ID NO: 101 - DNA, 22 bp, Artificial sequence
  DLX5 forward primer
acagagacttcacgactcccag

SEQ ID NO: 102 - DNA, 20 bp, Artificial sequence
  DLX5 reverse primer
tgtggggctgctctggtcta

SEQ ID NO: 103 - DNA, 25 bp, Artificial sequence
  DLX6 forward primer
tggtgaaagagaagcattttggact

SEQ ID NO: 104 - DNA, 24 bp, Artificial sequence
  DLX6 reverse primer
agagaagggctgttatgtgaggaa

SEQ ID NO: 105 - DNA, 20 bp, Artificial sequence
  SERT forward primer
tgctggcttttgctagctac

SEQ ID NO: 106 - DNA, 20 bp, Artificial sequence
  SERT reverse primer
gaagctcgtcatgcagttca

SEQ ID NO: 107 - DNA, 21 bp, Artificial sequence
  TPH2 forward primer
atggctcagatcccctctaca

SEQ ID NO: 108 - DNA, 21 bp, Artificial sequence
  TPH2 reverse primer
ggatccgcaagtagtggaaca

SEQ ID NO: 109 - DNA, 20 bp, Artificial sequence
  VGLUT1 forward primer
tcaagtccccgattccgtgc

SEQ ID NO: 110 - DNA, 22 bp, Artificial sequence
  VGLUT1 reverse primer
tgcgattttggttgtttcccca

SEQ ID NO: 111 - DNA, 20 bp, Artificial sequence
  VGLUT2 forward primer
tggggctacatcatcactca

SEQ ID NO: 112 - DNA, 20 bp, Artificial sequence
  VGLUT2 reverse primer
gaagtatggcagctccgaaa